European Patent Application EP 4 112 071 A1, published January 4, 2023. Title: NOVEL IMMUNIZATION AGENTS AND METHODS OF USE. Applicant: HSF PHARMACEUTICALS. Application EP 22164585.6, filed August 25, 2015. The sequence listing filed with the application follows.

SEQUENCE LISTING (26 sequences)

SEQ ID NO: 1 - DNA, 21 bp, Homo sapiens
  source 1..21: mol_type = other DNA
tcgacaactccgagtttcagc

SEQ ID NO: 2 - DNA, 39 bp, Homo sapiens
  source 1..39: mol_type = other DNA
ctcctcgcggccgcatcgatccatagagcccaccgcatc

SEQ ID NO: 3 - DNA, 42 bp, herpes simplex virus 1
  source 1..42: mol_type = other DNA
ctcctcaagcttctcgagcacacggagcgcggctgccgacac

SEQ ID NO: 4 - DNA, 35 bp, herpes simplex virus 1
  source 1..35: mol_type = other DNA
ctcctcggtaccccatggaggccagcagagccagc

SEQ ID NO: 5 - DNA, 42 bp, herpes simplex virus 1
  source 1..42: mol_type = other DNA
ctcctcgcggccgcactagttccgcgtgtccctttccgatgc

SEQ ID NO: 6 - DNA, 58 bp, herpes simplex virus 1
  source 1..58: mol_type = other DNA
ctcctcctcgagaagcttatgcatgagctcgacgtctcggcggtaatgagatacgagc

SEQ ID NO: 7 - DNA, 32 bp, herpes simplex virus 1
  source 1..32: mol_type = unassigned DNA
ctcctcagaacccaggaccagggccacgttgg

SEQ ID NO: 8 - DNA, 33 bp, herpes simplex virus 1
  source 1..33: mol_type = unassigned DNA
ctcctcatggagacaaagcccaagacggcaacc

SEQ ID NO: 9 - DNA, 36 bp, herpes simplex virus 1
  source 1..36: mol_type = unassigned DNA
ctcctcggagaccggggttggggaatgaatccctcc

SEQ ID NO: 10 - DNA, 35 bp, herpes simplex virus 1
  source 1..35: mol_type = unassigned DNA
ctcctcgcggggcgtgggaggggctggggcggacc

SEQ ID NO: 11 - DNA, 22 bp, herpes simplex virus 1
  source 1..22: mol_type = unassigned DNA
agagggacatccaggactttgt

SEQ ID NO: 12 - DNA, 19 bp, herpes simplex virus 1
  source 1..19: mol_type = unassigned DNA
caggcgcttgttggtgtac

SEQ ID NO: 13 - DNA, 16 bp, herpes simplex virus 1
  source 1..16: mol_type = unassigned DNA
accgccgaactgagca

SEQ ID NO: 14 - DNA, 15 bp, herpes simplex virus 1
  source 1..15: mol_type = unassigned DNA
cacgggccgcttcac

SEQ ID NO: 15 - DNA, 17 bp, herpes simplex virus 1
  source 1..17: mol_type = unassigned DNA
gcgatagcgcgcgtaga

SEQ ID NO: 16 - DNA, 14 bp, herpes simplex virus 1
  source 1..14: mol_type = unassigned DNA
ccgacgcgacctcc

SEQ ID NO: 17 - DNA, 17 bp, herpes simplex virus 1
  source 1..17: mol_type = unassigned DNA
cctccacgcccaaaagc

SEQ ID NO: 18 - DNA, 22 bp, herpes simplex virus 1
  source 1..22: mol_type = unassigned DNA
ggtggtgttgttcttgggtttg

SEQ ID NO: 19 - DNA, 15 bp, herpes simplex virus 1
  source 1..15: mol_type = unassigned DNA
ccccacgtccacccc

SEQ ID NO: 20 - DNA, 25 bp, Mus musculus
  source 1..25: mol_type = unassigned DNA
ctcaagaaatctaacccctgactca

SEQ ID NO: 21 - DNA, 16 bp, Mus musculus
  source 1..16: mol_type = unassigned DNA
gcgggacaggctgaga

SEQ ID NO: 22 - DNA, 15 bp, Mus musculus
  source 1..15: mol_type = unassigned DNA
ccccacacacacctc

SEQ ID NO: 23 - DNA, 27 bp, herpes simplex virus 1
  source 1..27: mol_type = unassigned DNA
gagctcatcaccgcaggcgagtctctt

SEQ ID NO: 24 - DNA, 27 bp, herpes simplex virus 1
  source 1..27: mol_type = unassigned DNA
gagctcggtcttcgggactaatgcctt

SEQ ID NO: 25 - DNA, 26 bp, herpes simplex virus 1
  source 1..26: mol_type = unassigned DNA
ggggtaccggttttgttttgtgtgac

SEQ ID NO: 26 - DNA, 26 bp, herpes simplex virus 1
  source 1..26: mol_type = unassigned DNA
ggggtaccggtgtgtgatgatttcgc